European Patent Application EP 4 446 339 A1, published October 16, 2024. Title: 识别RSV pre-F蛋白的抗体以及应用. Applicant: 厦门大学. Application CN. The sequence listing filed with the application follows.

SEQUENCE LISTING (63 sequences)

SEQ ID NO: 1 - protein, 574 aa, synthetic construct
  source 1..574: note = RSV A2 F protein
MELLILKANAITTILTAVTFCFASGQNITEEFYQSTCSAVSKGYLSALRTGWYTSVITIELSNIKKNKCNGTDAKIKLIKQELDKYKNAVTELQLLMQSTPATNNRARRELPRFMNYTLNNAKKTNVTLSKKRKRRFLGFLLGVGSAIASGVAVSKVLHLEGEVNKIKSALLSTNKAVVSLSNGVSVLTSKVLDLKNYIDKQLLPIVNKQSCSISNIETVIEFQQKNNRLLEITREFSVNAGVTTPVSTYMLTNSELLSLINDMPITNDQKKLMSNNVQIVRQQSYSIMSIIKEEVLAYVVQLPLYGVIDTPCWKLHTSPLCTTNTKEGSNICLTRTDRGWYCDNAGSVSFFPQAETCKVQSNRVFCDTMNSLTLPSEVNLCNVDIFNPKYDCKIMTSKTDVSSSVITSLGAIVSCYGKTKCTASNKNRGIIKTFSNGCDYVSNKGVDTVSVGNTLYYVNKQEGKSLYVKGEPIINFYDPLVFPSDEFDASISQVNEKINQSLAFIRKSDELLHNVNAVKSTTNIMITTIIIVIIVILLSLIAVGLLLYCKARSTPVTLSKDQLSGINNIAFSN

SEQ ID NO: 2 - DNA, 1725 bp, synthetic construct
  source 1..1725: mol_type = other DNA; note = nucleotide sequence encoding RSV A2 F protein
atggagttgctaatcctcaaagcaaatgcaattaccacaatcctcactgcagtcacattttgttttgcttctggtcaaaacatcactgaagaattttatcaatcaacatgcagtgcagttagcaaaggctatcttagtgctctgagaactggttggtataccagtgttataactatagaattaagtaatatcaagaaaaataagtgtaatggaacagatgctaaggtaaaattgataaaacaagaattagataaatataaaaatgctgtaacagaattgcagttgctcatgcaaagcacacaagcaacaaacaatcgagccagaagagaactaccaaggtttatgaattatacactcaacaatgccaaaaaaaccaatgtaacattaagcaagaaaaggaaaagaagatttcttggttttttgttaggtgttggatctgcaatcgccagtggcgttgctgtatctaaggtcctgcacctagaaggggaagtgaacaagatcaaaagtgctctactatccacaaacaaggctgtagtcagcttatcaaatggagttagtgttttaaccagcaaagtgttagacctcaaaaactatatagataaacaattgttacctattgtgaacaagcaaagctgcagcatatcaaatatagaaactgtgatagagttccaacaaaagaacaacagactactagagattaccagggaatttagtgttaatgcaggcgtaactacacctgtaagcacttacatgttaactaatagtgaattattgtcattaatcaatgatatgcctataacaaatgatcagaaaaagttaatgtccaacaatgttcaaatagttagacagcaaagttactctatcatgtccataataaaagaggaagtcttagcatatgtagtacaattaccactatatggtgttatagatacaccctgttggaaactacacacatcccctctatgtacaaccaacacaaaagaagggtccaacatctgtttaacaagaactgacagaggatggtactgtgacaatgcaggatcagtatctttcttcccacaagctgaaacatgtaaagttcaatcaaatcgagtattttgtgacacaatgaacagtttaacattaccaagtgaagtaaatctctgcaatgttgacatattcaaccccaaatatgattgtaaaattatgacttcaaaaacagatgtaagcagctccgttatcacatctctaggagccattgtgtcatgctatggcaaaactaaatgtacagcatccaataaaaatcgtggaatcataaagacattttctaacgggtgcgattatgtatcaaataaaggggtggacactgtgtctgtaggtaacacattatattatgtaaataagcaagaaggtaaaagtctctatgtaaaaggtgaaccaataataaatttctatgacccattagtattcccctctgatgaatttgatgcatcaatatctcaagtcaacgagaagattaaccagagcctagcatttattcgtaaatccgatgaattattacataatgtaaatgctggtaaatccaccacaaatatcatgataactactataattatagtgattatagtaatattgttatcattaattgctgttggactgctcttatactgtaaggccagaagcacaccagtcacactaagcaaagatcaactgagtggtataaataatattgcatttagtaactaa

SEQ ID NO: 3 - protein, 116 aa, synthetic construct
  source 1..116: note = 5B11 VH
QIQLVQSGPELKKPGETVKISCKASGYTFTDYSMHWLKQAPGKGLKWMGWITTETGEPTYADDFKGRFAFSLETSASTAYLQINNLKNEDTGIYFCARYYYGPFYWGQGTLVTVST

SEQ ID NO: 4 - protein, 107 aa, synthetic construct
  source 1..107: note = 5B11 VL
DIQMTQSPASLSASVGETVTITCRSSGNIHNFLTWYQQKQGKSPQFLVYNAKTLADGVSSRFSGSGSGTQFSLKINSLQPEDFGIYYCQHFWTTPYTFGGGTKLEIK

SEQ ID NO: 5 - protein, 8 aa, synthetic construct
  source 1..8: note = 5B11 VH CDR1
GYTFTDYS

SEQ ID NO: 6 - protein, 8 aa, synthetic construct
  source 1..8: note = 5B11 VH CDR2
ITTETGEP

SEQ ID NO: 7 - protein, 9 aa, synthetic construct
  source 1..9: note = 5B11 VH CDR3
ARYYYGPFY

SEQ ID NO: 8 - protein, 6 aa, synthetic construct
  source 1..6: note = 5B11 VL CDR1
GNIHNF

SEQ ID NO: 9 - skipped

SEQ ID NO: 10 - protein, 9 aa, synthetic construct
  source 1..9: note = 5B11 VL CDR3
QHFWTTPYT

SEQ ID NO: 11 - protein, 119 aa, synthetic construct
  source 1..119: note = 6B2 VH
EVQLQQSRPELVKPGASVKISCKASGYSFTAYFMNWVKQSHGKSLEWIGRINPYIGDTFYNQKFKGKATLTVDKSSNTAHMELLSLTSEDSAVYYCGRSEYGNYYFDYWGQGTTLTVSQ

SEQ ID NO: 12 - protein, 106 aa, synthetic construct
  source 1..106: note = 6B2 VL
ENVLTQSPAIMSASLGEKVTMSCRASSSVNYMYWYQQKSDASPKLWIYYTSNLAPGVPARFSGSGSGNSYSLTISSMEGEDAATYYCQQFTSSPLTFGAGTKLELK

SEQ ID NO: 13 - protein, 8 aa, synthetic construct
  source 1..8: note = 6B2 VH CDR1
GYSFTAYF

SEQ ID NO: 14 - protein, 8 aa, synthetic construct
  source 1..8: note = 6B2 VH CDR2
INPYIGDT

SEQ ID NO: 15 - protein, 12 aa, synthetic construct
  source 1..12: note = 6B2 VH CDR3
GRSEYGNYYFDY

SEQ ID NO: 16 - protein, 5 aa, synthetic construct
  source 1..5: note = 6B2 VL CDR1
SSVNY

SEQ ID NO: 17 - skipped

SEQ ID NO: 18 - protein, 9 aa, synthetic construct
  source 1..9: note = 6B2 VL CDR3
QQFTSSPLT

SEQ ID NO: 19 - protein, 118 aa, synthetic construct
  source 1..118: note = 7G5 VH
QVQLKESGPGLVAPSQSLSITCTVSGFSLSSYGVHWIRQPPGKGLEWLGVIWAGGSTNYNSALMSRLSISEDNSKSQVFLKMNSLQTDDTAVYYCARKGLVWPAMDYWGQGTSVTVSQ

SEQ ID NO: 20 - protein, 107 aa, synthetic construct
  source 1..107: note = 7G5 VL
DIQMTQTTSSLSASLGDRVTISCRASQDISHYLNWYQQKPDGTVKLLIYYTSRLHSGVPSRFSGSGSGTDYSLTIYNLEQEDIATYFCQQGNTLPWTFGGGTKLEIK

SEQ ID NO: 21 - protein, 8 aa, synthetic construct
  source 1..8: note = 7G5 VH CDR1
GFSLSSYG

SEQ ID NO: 22 - protein, 7 aa, synthetic construct
  source 1..7: note = 7G5 VH CDR2
IWAGGST

SEQ ID NO: 23 - protein, 12 aa, synthetic construct
  source 1..12: note = 7G5 VH CDR3
ARKGLVWPAMDY

SEQ ID NO: 24 - protein, 6 aa, synthetic construct
  source 1..6: note = 7G5 VL CDR1
QDISHY

SEQ ID NO: 25 - skipped

SEQ ID NO: 26 - protein, 9 aa, synthetic construct
  source 1..9: note = 7G5 VL CDR3
QQGNTLPWT

SEQ ID NO: 27 - DNA, 25 bp, synthetic construct
  source 1..25: mol_type = other DNA; note = primer MVJkR
ccgtttgkatytccagcttggtscc

SEQ ID NO: 28 - DNA, 25 bp, synthetic construct
  source 1..25: mol_type = other DNA; note = primer MVDJhR
cggtgaccgwggtbccttgrcccca

SEQ ID NO: 29 - DNA, 33 bp, synthetic construct
  source 1..33: mol_type = other DNA; note = primer MuIgVH5'-A
gggaattcatgrasttskggytmarctkgrttt

SEQ ID NO: 30 - DNA, 34 bp, synthetic construct
  source 1..34: mol_type = other DNA; note = primer MuIgVH5'-B
gggaattcatgraatgsasctgggtywtyctctt

SEQ ID NO: 31 - DNA, 39 bp, synthetic construct
  source 1..39: mol_type = other DNA; note = primer MuIgVH5'-C1
actagtcgacatggactccaggctcaatttagttttcct

SEQ ID NO: 32 - DNA, 36 bp, synthetic construct
  source 1..36: mol_type = other DNA; note = primer MuIgVH5'-C2
actagtcgacatggctgtcytrgbgctgytcytctg

SEQ ID NO: 33 - DNA, 39 bp, synthetic construct
  source 1..39: mol_type = other DNA; note = primer MuIgVH5'-C3
actagtcgacatggvttggstgtggamcttgcyattcct

SEQ ID NO: 34 - DNA, 36 bp, synthetic construct
  source 1..36: mol_type = other DNA; note = primer MuIgVH5'-D1
actagtcgacatgaaatgcagctggrtyatsttctt

SEQ ID NO: 35 - DNA, 36 bp, synthetic construct
  source 1..36: mol_type = other DNA; note = primer MuIgVH5'-D2
actagtcgacatggrcagrcttacwtyytcattcct

SEQ ID NO: 36 - DNA, 36 bp, synthetic construct
  source 1..36: mol_type = other DNA; note = primer MuIgVH5'-D3
actagtcgacatgatggtgttaagtcttctgtacct

SEQ ID NO: 37 - DNA, 36 bp, synthetic construct
  source 1..36: mol_type = other DNA; note = primer MuIgVH5'-E1
actagtcgacatgggatggagctrtatcatsytctt

SEQ ID NO: 38 - DNA, 33 bp, synthetic construct
  source 1..33: mol_type = other DNA; note = primer MuIgVH5'-E2
actagtcgacatgaagwtgtggbtraactggrt

SEQ ID NO: 39 - DNA, 35 bp, synthetic construct
  source 1..35: mol_type = other DNA; note = primer MuIgVH5'-E3
  misc_feature 25: note = n represents hypoxanthine deoxyribonucleotide residue
actagtcgacatggratggasckknrtctttmtct

SEQ ID NO: 40 - DNA, 35 bp, synthetic construct
  source 1..35: mating_type = primer MuIgVH5'-F1; mol_type = other DNA
actagtcgacatgaacttygggytsagmttgrttt

SEQ ID NO: 41 - DNA, 35 bp, synthetic construct
  source 1..35: mol_type = other DNA; note = primer MuIgVH5'-F2
actagtcgacatgtacttgggactgagctgtgtat

SEQ ID NO: 42 - DNA, 33 bp, synthetic construct
  source 1..33: mol_type = other DNA; note = primer MuIgVH5'-F3
actagtcgacatgagagtgctgattcttttgtg

SEQ ID NO: 43 - DNA, 38 bp, synthetic construct
  source 1..38: mol_type = other DNA; note = primer MuIgVH5'-F4
actagtcgacatggattttgggctgattttttttattg

SEQ ID NO: 44 - DNA, 32 bp, synthetic construct
  source 1..32: mol_type = other DNA; note = primer MuIgkappaVL5'-A
gggaattcatgragwcacakwcycaggtcttt

SEQ ID NO: 45 - DNA, 33 bp, synthetic construct
  source 1..33: mol_type = other DNA; note = primer MuIgkappaVL5'-B
gggaattcatggagacagacacactcctgctat

SEQ ID NO: 46 - DNA, 39 bp, synthetic construct
  source 1..39: mol_type = other DNA; note = primer MuIgkappaVL5'-C
actagtcgacatggagwcagacacactsctgytatgggt

SEQ ID NO: 47 - DNA, 42 bp, synthetic construct
  source 1..42: mol_type = other DNA; note = primer MuIgkappaVL5'-D1
  misc_feature 37: note = n represents hypoxanthine deoxyribonucleotide residue
actagtcgacatgaggrcccctgctcagwttyttggnwtctt

SEQ ID NO: 48 - DNA, 41 bp, synthetic construct
  source 1..41: mol_type = other DNA; note = primer MuIgkappaVL5'-D2
actagtcgacatgggcwtcaagatgragtcacakwyycwgg

SEQ ID NO: 49 - DNA, 39 bp, synthetic construct
  source 1..39: mol_type = other DNA; note = primer MuIgkappaVL5'-E1
actagtcgacatgagtgtgcycactcaggtcctggsgtt

SEQ ID NO: 50 - DNA, 41 bp, synthetic construct
  source 1..41: mol_type = other DNA; note = primer MuIgkappaVL5'-E2
actagtcgacatgtggggaycgktttyammcttttcaattg

SEQ ID NO: 51 - DNA, 38 bp, synthetic construct
  source 1..38: mol_type = other DNA; note = primer MuIgkappaVL5'-E3
actagtcgacatggaagccccagctcagcttctcttcc

SEQ ID NO: 52 - DNA, 36 bp, synthetic construct
  source 1..36: mol_type = other DNA; note = primer MuIgkappaVL5'-F1
  misc_feature 16: note = n represents hypoxanthine deoxyribonucleotide residue
  misc_feature 22: note = n represents hypoxanthine deoxyribonucleotide residue
  misc_feature 28: note = n represents hypoxanthine deoxyribonucleotide residue
actagtcgacatgagnmmktcnmttcanttcytggg

SEQ ID NO: 53 - DNA, 36 bp, synthetic construct
  source 1..36: mol_type = other DNA; note = primer MuIgkappaVL5'-F2
  misc_feature 22: note = n represents hypoxanthine deoxyribonucleotide residue
  misc_feature 34: map = n represents hypoxanthine deoxyribonucleotide residue
actagtcgacatgakgthcycngctcagytyctnrg

SEQ ID NO: 54 - DNA, 35 bp, synthetic construct
  source 1..35: mol_type = other DNA; note = primer MuIgkappaVL5'-F3
actagtcgacatggtrtccwcasctcagttccttg

SEQ ID NO: 55 - DNA, 37 bp, synthetic construct
  source 1..37: mol_type = other DNA; note = primer MuIgkappaVL5'-F4
actagtcgacatgtatatatgtttgttgtctatttct

SEQ ID NO: 56 - DNA, 39 bp, synthetic construct
  source 1..39: mol_type = other DNA; note = primer MuIgkappaVL5'-G1
actagtcgacatgaagttgcctgttaggctgttggtgct

SEQ ID NO: 57 - DNA, 39 bp, synthetic construct
  source 1..39: mol_type = other DNA; note = primer MuIgkappaVL5'-G2
actagtcgacatggatttwcargtgcagattwtcagctt

SEQ ID NO: 58 - DNA, 37 bp, synthetic construct
  source 1..37: mol_type = other DNA; note = primer MuIgkappaVL5'-G3
actagtcgacatggtyctyatvtccttgctgttctgg

SEQ ID NO: 59 - DNA, 37 bp, synthetic construct
  source 1..37: mol_type = other DNA; note = primer MuIgkappaVL5'-G4
actagtcgacatggtyctyatvttrctgctgctatgg

SEQ ID NO: 60 - protein, 116 aa, synthetic construct
  source 1..116: note = N5B11 VH
QIQLVQSGPELKKPGASVKISCKASGYTFTDYSMHWLKQAPGKGLKWMGWITTETGEPTYADDFKGRFAFSLDTSASTAYLQISSLKAEDTGVYFCARYYYGPFYWGQGTLVTVSS

SEQ ID NO: 61 - protein, 107 aa, synthetic construct
  source 1..107: note = N5B11 VL
DIQMTQSPSSLSASVGDRVTITCRSSGNIHNFLTWYQQKPGKSPQFLVYNAKTLADGVPSRFSGSGSGTQFTLTISSLQPEDFGIYYCQHFWTTPYTFGGGTKVEIK

SEQ ID NO: 62 - protein, 330 aa, synthetic construct [sequence omitted]

SEQ ID NO: 63 - protein, 107 aa, synthetic construct [sequence omitted]